European Patent Application EP 4 218 795 A2, published August 2, 2023. Title: PTH compounds with low peak-to-trough ratios. Applicant: Ascendis Pharma Bone Diseases A/S. Application EP, filed February 20, 2023. The sequence listing filed with the application follows.

SEQUENCE LISTING (122 sequences)

SEQ ID NO: 1 - protein, 84 aa, Homo sapiens
SVSEIQLMHNLGKHLNSMERVEWLRKKLQDVHNFVALGAPLAPRDAGSQRPRKKEDNVLVESHEKSLGEADKADVNVLTKAKSQ

SEQ ID NO: 2 - protein, 83 aa, synthetic construct
  REGION 1..83: note = Human PTH 1-83
SVSEIQLMHNLGKHLNSMERVEWLRKKLQDVHNFVALGAPLAPRDAGSQRPRKKEDNVLVESHEKSLGEADKADVNVLTKAKS

SEQ ID NO: 3 - protein, 82 aa, synthetic construct
  REGION 1..82: note = human PTH 1-82
SVSEIQLMHNLGKHLNSMERVEWLRKKLQDVHNFVALGAPLAPRDAGSQRPRKKEDNVLVESHEKSLGEADKADVNVLTKAK

SEQ ID NO: 4 - protein, 81 aa, synthetic construct
  REGION 1..81: note = human PTH 1-81
SVSEIQLMHNLGKHLNSMERVEWLRKKLQDVHNFVALGAPLAPRDAGSQRPRKKEDNVLVESHEKSLGEADKADVNVLTKA

SEQ ID NO: 5 - protein, 80 aa, synthetic construct
  REGION 1..80: note = human PTH 1-80
SVSEIQLMHNLGKHLNSMERVEWLRKKLQDVHNFVALGAPLAPRDAGSQRPRKKEDNVLVESHEKSLGEADKADVNVLTK

SEQ ID NO: 6 - protein, 79 aa, synthetic construct
  REGION 1..79: note = human PTH 1-79
SVSEIQLMHNLGKHLNSMERVEWLRKKLQDVHNFVALGAPLAPRDAGSQRPRKKEDNVLVESHEKSLGEADKADVNVLT

SEQ ID NO: 7 - protein, 78 aa, synthetic construct
  REGION 1..78: note = human PTH 1-78
SVSEIQLMHNLGKHLNSMERVEWLRKKLQDVHNFVALGAPLAPRDAGSQRPRKKEDNVLVESHEKSLGEADKADVNVL

SEQ ID NO: 8 - protein, 77 aa, synthetic construct
  REGION 1..77: note = human PTH 1-77
SVSEIQLMHNLGKHLNSMERVEWLRKKLQDVHNFVALGAPLAPRDAGSQRPRKKEDNVLVESHEKSLGEADKADVNV

SEQ ID NO: 9 - protein, 76 aa, synthetic construct
  REGION 1..76: note = human PTH 1-76
SVSEIQLMHNLGKHLNSMERVEWLRKKLQDVHNFVALGAPLAPRDAGSQRPRKKEDNVLVESHEKSLGEADKADVN

SEQ ID NO: 10 - protein, 75 aa, synthetic construct
  REGION 1..75: note = human PTH 1-75
SVSEIQLMHNLGKHLNSMERVEWLRKKLQDVHNFVALGAPLAPRDAGSQRPRKKEDNVLVESHEKSLGEADKADV

SEQ ID NO: 11 - protein, 74 aa, synthetic construct
  REGION 1..74: note = human PTH 1-74
SVSEIQLMHNLGKHLNSMERVEWLRKKLQDVHNFVALGAPLAPRDAGSQRPRKKEDNVLVESHEKSLGEADKAD

SEQ ID NO: 12 - protein, 73 aa, synthetic construct
  REGION 1..73: note = human PTH 1-73
SVSEIQLMHNLGKHLNSMERVEWLRKKLQDVHNFVALGAPLAPRDAGSQRPRKKEDNVLVESHEKSLGEADKA

SEQ ID NO: 13 - protein, 72 aa, synthetic construct
  REGION 1..72: note = human PTH 1-72
SVSEIQLMHNLGKHLNSMERVEWLRKKLQDVHNFVALGAPLAPRDAGSQRPRKKEDNVLVESHEKSLGEADK

SEQ ID NO: 14 - protein, 71 aa, synthetic construct
  REGION 1..71: note = human PTH 1-71
SVSEIQLMHNLGKHLNSMERVEWLRKKLQDVHNFVALGAPLAPRDAGSQRPRKKEDNVLVESHEKSLGEAD

SEQ ID NO: 15 - protein, 70 aa, synthetic construct
  REGION 1..70: note = human PTH 1-70
SVSEIQLMHNLGKHLNSMERVEWLRKKLQDVHNFVALGAPLAPRDAGSQRPRKKEDNVLVESHEKSLGEA

SEQ ID NO: 16 - protein, 69 aa, synthetic construct
  REGION 1..69: note = human PTH 1-69
SVSEIQLMHNLGKHLNSMERVEWLRKKLQDVHNFVALGAPLAPRDAGSQRPRKKEDNVLVESHEKSLGE

SEQ ID NO: 17 - protein, 68 aa, synthetic construct
  REGION 1..68: note = human PTH 1-68
SVSEIQLMHNLGKHLNSMERVEWLRKKLQDVHNFVALGAPLAPRDAGSQRPRKKEDNVLVESHEKSLG

SEQ ID NO: 18 - protein, 67 aa, synthetic construct
  REGION 1..67: note = human PTH 1-67
SVSEIQLMHNLGKHLNSMERVEWLRKKLQDVHNFVALGAPLAPRDAGSQRPRKKEDNVLVESHEKSL

SEQ ID NO: 19 - protein, 66 aa, synthetic construct
  REGION 1..66: note = human PTH 1-66
SVSEIQLMHNLGKHLNSMERVEWLRKKLQDVHNFVALGAPLAPRDAGSQRPRKKEDNVLVESHEKS

SEQ ID NO: 20 - protein, 65 aa, synthetic construct
  REGION 1..65: note = human PTH 1-65
SVSEIQLMHNLGKHLNSMERVEWLRKKLQDVHNFVALGAPLAPRDAGSQRPRKKEDNVLVESHEK

SEQ ID NO: 21 - protein, 64 aa, synthetic construct
  REGION 1..64: note = human PTH 1-64
SVSEIQLMHNLGKHLNSMERVEWLRKKLQDVHNFVALGAPLAPRDAGSQRPRKKEDNVLVESHE

SEQ ID NO: 22 - protein, 63 aa, synthetic construct
  REGION 1..63: note = human PTH 1-63
SVSEIQLMHNLGKHLNSMERVEWLRKKLQDVHNFVALGAPLAPRDAGSQRPRKKEDNVLVESH

SEQ ID NO: 23 - protein, 62 aa, synthetic construct
  REGION 1..62: note = human PTH 1-62
SVSEIQLMHNLGKHLNSMERVEWLRKKLQDVHNFVALGAPLAPRDAGSQRPRKKEDNVLVES

SEQ ID NO: 24 - protein, 61 aa, synthetic construct
  REGION 1..61: note = human PTH 1-61
SVSEIQLMHNLGKHLNSMERVEWLRKKLQDVHNFVALGAPLAPRDAGSQRPRKKEDNVLVE

SEQ ID NO: 25 - protein, 60 aa, synthetic construct
  REGION 1..60: note = human PTH 1-60
SVSEIQLMHNLGKHLNSMERVEWLRKKLQDVHNFVALGAPLAPRDAGSQRPRKKEDNVLV

SEQ ID NO: 26 - protein, 59 aa, synthetic construct
  REGION 1..59: note = human PTH 1-59
SVSEIQLMHNLGKHLNSMERVEWLRKKLQDVHNFVALGAPLAPRDAGSQRPRKKEDNVL

SEQ ID NO: 27 - protein, 58 aa, synthetic construct
  REGION 1..58: note = human PTH 1-58
SVSEIQLMHNLGKHLNSMERVEWLRKKLQDVHNFVALGAPLAPRDAGSQRPRKKEDNV

SEQ ID NO: 28 - protein, 57 aa, synthetic construct
  REGION 1..57: note = human PTH 1-57
SVSEIQLMHNLGKHLNSMERVEWLRKKLQDVHNFVALGAPLAPRDAGSQRPRKKEDN

SEQ ID NO: 29 - protein, 56 aa, synthetic construct
  REGION 1..56: note = human PTH 1-56
SVSEIQLMHNLGKHLNSMERVEWLRKKLQDVHNFVALGAPLAPRDAGSQRPRKKED

SEQ ID NO: 30 - protein, 55 aa, synthetic construct
  REGION 1..55: note = human PTH 1-55
SVSEIQLMHNLGKHLNSMERVEWLRKKLQDVHNFVALGAPLAPRDAGSQRPRKKE

SEQ ID NO: 31 - protein, 54 aa, synthetic construct
  REGION 1..54: note = human PTH 1-54
SVSEIQLMHNLGKHLNSMERVEWLRKKLQDVHNFVALGAPLAPRDAGSQRPRKK

SEQ ID NO: 32 - protein, 53 aa, synthetic construct
  REGION 1..53: note = human PTH 1-53
SVSEIQLMHNLGKHLNSMERVEWLRKKLQDVHNFVALGAPLAPRDAGSQRPRK

SEQ ID NO: 33 - protein, 52 aa, synthetic construct
  REGION 1..52: note = human PTH 1-52
SVSEIQLMHNLGKHLNSMERVEWLRKKLQDVHNFVALGAPLAPRDAGSQRPR

SEQ ID NO: 34 - protein, 51 aa, synthetic construct
  REGION 1..51: note = human PTH 1-51
SVSEIQLMHNLGKHLNSMERVEWLRKKLQDVHNFVALGAPLAPRDAGSQRP

SEQ ID NO: 35 - protein, 50 aa, synthetic construct
  REGION 1..50: note = human PTH 1-50
SVSEIQLMHNLGKHLNSMERVEWLRKKLQDVHNFVALGAPLAPRDAGSQR

SEQ ID NO: 36 - protein, 49 aa, synthetic construct
  REGION 1..49: note = human PTH 1-49
SVSEIQLMHNLGKHLNSMERVEWLRKKLQDVHNFVALGAPLAPRDAGSQ

SEQ ID NO: 37 - protein, 48 aa, synthetic construct
  REGION 1..48: note = human PTH 1-48
SVSEIQLMHNLGKHLNSMERVEWLRKKLQDVHNFVALGAPLAPRDAGS

SEQ ID NO: 38 - protein, 47 aa, synthetic construct
  REGION 1..47: note = human PTH 1-47
SVSEIQLMHNLGKHLNSMERVEWLRKKLQDVHNFVALGAPLAPRDAG

SEQ ID NO: 39 - protein, 46 aa, synthetic construct
  REGION 1..46: note = human PTH 1-46
SVSEIQLMHNLGKHLNSMERVEWLRKKLQDVHNFVALGAPLAPRDA

SEQ ID NO: 40 - protein, 45 aa, synthetic construct
  REGION 1..45: note = human PTH 1-45
SVSEIQLMHNLGKHLNSMERVEWLRKKLQDVHNFVALGAPLAPRD

SEQ ID NO: 41 - protein, 44 aa, synthetic construct
  REGION 1..44: note = human PTH 1-44
SVSEIQLMHNLGKHLNSMERVEWLRKKLQDVHNFVALGAPLAPR

SEQ ID NO: 42 - protein, 43 aa, synthetic construct
  REGION 1..43: note = human PTH 1-43
SVSEIQLMHNLGKHLNSMERVEWLRKKLQDVHNFVALGAPLAP

SEQ ID NO: 43 - protein, 42 aa, synthetic construct
  REGION 1..42: note = human PTH 1-42
SVSEIQLMHNLGKHLNSMERVEWLRKKLQDVHNFVALGAPLA

SEQ ID NO: 44 - protein, 41 aa, synthetic construct
  REGION 1..41: note = human PTH-41
SVSEIQLMHNLGKHLNSMERVEWLRKKLQDVHNFVALGAPL

SEQ ID NO: 45 - protein, 40 aa, synthetic construct
  REGION 1..40: note = human PTH 1-40
SVSEIQLMHNLGKHLNSMERVEWLRKKLQDVHNFVALGAP

SEQ ID NO: 46 - protein, 39 aa, synthetic construct
  REGION 1..39: note = human PTH 1-39
SVSEIQLMHNLGKHLNSMERVEWLRKKLQDVHNFVALGA

SEQ ID NO: 47 - protein, 38 aa, synthetic construct
  REGION 1..38: note = human PTH 1-38
SVSEIQLMHNLGKHLNSMERVEWLRKKLQDVHNFVALG

SEQ ID NO: 48 - protein, 37 aa, synthetic construct
  REGION 1..37: note = human PTH 1-37
SVSEIQLMHNLGKHLNSMERVEWLRKKLQDVHNFVAL

SEQ ID NO: 49 - protein, 36 aa, synthetic construct
  REGION 1..36: note = human PTH 1-36
SVSEIQLMHNLGKHLNSMERVEWLRKKLQDVHNFVA

SEQ ID NO: 50 - protein, 35 aa, synthetic construct
  REGION 1..35: note = human PTH 1-35
SVSEIQLMHNLGKHLNSMERVEWLRKKLQDVHNFV

SEQ ID NO: 51 - protein, 34 aa, synthetic construct
  REGION 1..34: note = human PTH 1-34
SVSEIQLMHNLGKHLNSMERVEWLRKKLQDVHNF

SEQ ID NO: 52 - protein, 33 aa, synthetic construct
  REGION 1..33: note = human PTH 1-33
SVSEIQLMHNLGKHLNSMERVEWLRKKLQDVHN

SEQ ID NO: 53 - protein, 32 aa, synthetic construct
  REGION 1..32: note = human PTH 1-32
SVSEIQLMHNLGKHLNSMERVEWLRKKLQDVH

SEQ ID NO: 54 - protein, 31 aa, synthetic construct
  REGION 1..31: note = human PTH 1-31
SVSEIQLMHNLGKHLNSMERVEWLRKKLQDV

SEQ ID NO: 55 - protein, 30 aa, synthetic construct
  REGION 1..30: note = human PTH 1-30
SVSEIQLMHNLGKHLNSMERVEWLRKKLQD

SEQ ID NO: 56 - protein, 29 aa, synthetic construct
  REGION 1..29: note = human PTH 1-29
SVSEIQLMHNLGKHLNSMERVEWLRKKLQ

SEQ ID NO: 57 - protein, 28 aa, synthetic construct
  REGION 1..28: note = human PTH 1-28
SVSEIQLMHNLGKHLNSMERVEWLRKKL

SEQ ID NO: 58 - protein, 27 aa, synthetic construct
  REGION 1..27: note = human PTH 1-27
SVSEIQLMHNLGKHLNSMERVEWLRKK

SEQ ID NO: 59 - protein, 26 aa, synthetic construct
  REGION 1..26: note = human PTH 1-26
SVSEIQLMHNLGKHLNSMERVEWLRK

SEQ ID NO: 60 - protein, 25 aa, synthetic construct
  REGION 1..25: note = human PTH 1-25
SVSEIQLMHNLGKHLNSMERVEWLR

SEQ ID NO: 61 - protein, 84 aa, synthetic construct; identical to SEQ ID NO: 1
  REGION 1..84: note = amidated human PTH 1-84
  MOD_RES 84: note = AMIDATION

SEQ ID NO: 62 - protein, 83 aa, synthetic construct; identical to SEQ ID NO: 2
  REGION 1..83: note = amidated human PTH 1-83
  MOD_RES 83: note = AMIDATION

SEQ ID NO: 63 - protein, 82 aa, synthetic construct; identical to SEQ ID NO: 3
  REGION 1..82: note = amidated human PTH 1-82
  MOD_RES 82: note = AMIDATION

SEQ ID NO: 64 - protein, 81 aa, synthetic construct; identical to SEQ ID NO: 4
  REGION 1..81: note = amidated human PTH 1-81
  MOD_RES 81: note = AMIDATION

SEQ ID NO: 65 - protein, 80 aa, synthetic construct; identical to SEQ ID NO: 5
  REGION 1..80: note = amidated human PTH 1-80
  MOD_RES 80: note = AMIDATION

SEQ ID NO: 66 - protein, 79 aa, synthetic construct; identical to SEQ ID NO: 6
  REGION 1..79: note = amidated human PTH 1-79
  MOD_RES 79: note = AMIDATION

SEQ ID NO: 67 - protein, 78 aa, synthetic construct; identical to SEQ ID NO: 7
  REGION 1..78: note = amidated human PTH 1-78
  MOD_RES 78: note = AMIDATION

SEQ ID NO: 68 - protein, 77 aa, synthetic construct; identical to SEQ ID NO: 8
  REGION 1..77: note = amidated human PTH 1-77
  MOD_RES 77: note = AMIDATION

SEQ ID NO: 69 - protein, 76 aa, synthetic construct; identical to SEQ ID NO: 9
  REGION 1..76: note = amidated human PTH 1-76
  MOD_RES 76: note = AMIDATION

SEQ ID NO: 70 - protein, 75 aa, synthetic construct; identical to SEQ ID NO: 10
  REGION 1..75: note = amidated human PTH 1-75
  MOD_RES 75: note = AMIDATION

SEQ ID NO: 71 - protein, 74 aa, synthetic construct; identical to SEQ ID NO: 11
  REGION 1..74: note = amidated human PTH 1-74
  MOD_RES 74: note = AMIDATION

SEQ ID NO: 72 - protein, 73 aa, synthetic construct; identical to SEQ ID NO: 12
  REGION 1..73: note = amidated human PTH 1-73
  MOD_RES 73: note = AMIDATION

SEQ ID NO: 73 - protein, 72 aa, synthetic construct; identical to SEQ ID NO: 13
  REGION 1..72: note = amidated human PTH 1-72
  MOD_RES 72: note = AMIDATION

SEQ ID NO: 74 - protein, 71 aa, synthetic construct; identical to SEQ ID NO: 14
  REGION 1..71: note = amidated human PTH 1-71
  MOD_RES 71: note = AMIDATION

SEQ ID NO: 75 - protein, 70 aa, synthetic construct; identical to SEQ ID NO: 15
  REGION 1..70: note = amidated human PTH 1-70
  MOD_RES 70: note = AMIDATION

SEQ ID NO: 76 - protein, 69 aa, synthetic construct; identical to SEQ ID NO: 16
  REGION 1..69: note = amidated human PTH 1-69
  MOD_RES 69: note = AMIDATION

SEQ ID NO: 77 - protein, 68 aa, synthetic construct; identical to SEQ ID NO: 17
  REGION 1..68: note = amidated human PTH 1-68
  MOD_RES 68: note = AMIDATION

SEQ ID NO: 78 - protein, 67 aa, synthetic construct; identical to SEQ ID NO: 18
  REGION 1..67: note = amidated human PTH 1-67
  MOD_RES 67: note = AMIDATION

SEQ ID NO: 79 - protein, 66 aa, synthetic construct; identical to SEQ ID NO: 19
  REGION 1..66: note = amidated human PTH 1-66
  MOD_RES 66: note = AMIDATION

SEQ ID NO: 80 - protein, 65 aa, synthetic construct; identical to SEQ ID NO: 20
  REGION 1..65: note = amidated human PTH 1-65
  MOD_RES 65: note = AMIDATION

SEQ ID NO: 81 - protein, 64 aa, synthetic construct; identical to SEQ ID NO: 21
  REGION 1..64: note = amidated human PTH 1-64
  MOD_RES 64: note = AMIDATION

SEQ ID NO: 82 - protein, 63 aa, synthetic construct; identical to SEQ ID NO: 22
  REGION 1..63: note = amidated human PTH 1-63
  MOD_RES 63: note = AMIDATION

SEQ ID NO: 83 - protein, 62 aa, synthetic construct; identical to SEQ ID NO: 23
  REGION 1..62: note = amidated human PTH 1-62
  MOD_RES 62: note = AMIDATION

SEQ ID NO: 84 - protein, 61 aa, synthetic construct; identical to SEQ ID NO: 24
  REGION 1..61: note = amidated human PTH 1-61
  MOD_RES 61: note = AMIDATION

SEQ ID NO: 85 - protein, 60 aa, synthetic construct; identical to SEQ ID NO: 25
  REGION 1..60: note = amidated human PTH 1-60
  MOD_RES 60: note = ACETYLATION

SEQ ID NO: 86 - protein, 59 aa, synthetic construct; identical to SEQ ID NO: 26
  REGION 1..59: note = amidated human PTH 1-59
  MOD_RES 59: note = AMIDATION

SEQ ID NO: 87 - protein, 58 aa, synthetic construct; identical to SEQ ID NO: 27
  REGION 1..58: note = amidated human PTH 1-58
  MOD_RES 58: note = AMIDATION

SEQ ID NO: 88 - protein, 57 aa, synthetic construct; identical to SEQ ID NO: 28
  REGION 1..57: note = amidated human PTH 1-57
  MOD_RES 57: note = AMIDATION

SEQ ID NO: 89 - protein, 56 aa, synthetic construct; identical to SEQ ID NO: 29
  REGION 1..56: note = amidated human PTH 1-56
  MOD_RES 56: note = AMIDATION

SEQ ID NO: 90 - protein, 55 aa, synthetic construct; identical to SEQ ID NO: 30
  REGION 1..55: note = amidated human PTH 1-55
  MOD_RES 55: note = AMIDATION

SEQ ID NO: 91 - protein, 54 aa, synthetic construct; identical to SEQ ID NO: 31
  REGION 1..54: note = amidated human PTH 1-54
  MOD_RES 54: note = AMIDATION

SEQ ID NO: 92 - protein, 53 aa, synthetic construct; identical to SEQ ID NO: 32
  REGION 1..53: note = amidated human PTH 1-53
  MOD_RES 53: note = AMIDATION

SEQ ID NO: 93 - protein, 52 aa, synthetic construct; identical to SEQ ID NO: 33
  REGION 1..52: note = amidated human PTH 1-52
  MOD_RES 52: note = AMIDATION

SEQ ID NO: 94 - protein, 51 aa, synthetic construct; identical to SEQ ID NO: 34
  REGION 1..51: note = amidated human PTH 1-51
  MOD_RES 51: note = AMIDATION

SEQ ID NO: 95 - protein, 50 aa, synthetic construct; identical to SEQ ID NO: 35
  REGION 1..50: note = amidated human PTH 1-50
  MOD_RES 50: note = AMIDATION

SEQ ID NO: 96 - protein, 49 aa, synthetic construct; identical to SEQ ID NO: 36
  REGION 1..49: note = amidated human PTH 1-49
  MOD_RES 49: note = AMIDATION

SEQ ID NO: 97 - protein, 48 aa, synthetic construct; identical to SEQ ID NO: 37
  REGION 1..48: note = amidated human PTH 1-48
  MOD_RES 48: note = AMIDATION

SEQ ID NO: 98 - protein, 47 aa, synthetic construct; identical to SEQ ID NO: 38
  REGION 1..47: note = amidated human PTH 1-47
  MOD_RES 47: note = AMIDATION

SEQ ID NO: 99 - protein, 46 aa, synthetic construct; identical to SEQ ID NO: 39
  REGION 1..46: note = amidated human PTH 1-46
  MOD_RES 46: note = AMIDATION

SEQ ID NO: 100 - protein, 45 aa, synthetic construct; identical to SEQ ID NO: 40
  REGION 1..45: note = amidated human PTH 1-45
  MOD_RES 45: note = AMIDATION

SEQ ID NO: 101 - protein, 44 aa, synthetic construct; identical to SEQ ID NO: 41
  REGION 1..44: note = amidated human PTH 1-44
  MOD_RES 44: note = AMIDATION

SEQ ID NO: 102 - protein, 43 aa, synthetic construct; identical to SEQ ID NO: 42
  REGION 1..43: note = amidated human PTH 1-43
  MOD_RES 43: note = AMIDATION

SEQ ID NO: 103 - protein, 42 aa, synthetic construct; identical to SEQ ID NO: 43
  REGION 1..42: note = amidated human PTH 1-42
  MOD_RES 42: note = AMIDATION

SEQ ID NO: 104 - protein, 41 aa, synthetic construct; identical to SEQ ID NO: 44
  REGION 1..41: note = amidated human PTH 1-41
  MOD_RES 41: note = AMIDATION

SEQ ID NO: 105 - protein, 40 aa, synthetic construct; identical to SEQ ID NO: 45
  REGION 1..40: note = amidated human PTH 1-40
  MOD_RES 40: note = AMIDATION

SEQ ID NO: 106 - protein, 39 aa, synthetic construct; identical to SEQ ID NO: 46
  REGION 1..39: note = amidated human PTH 1-39
  MOD_RES 39: note = AMIDATION

SEQ ID NO: 107 - protein, 38 aa, synthetic construct; identical to SEQ ID NO: 47
  REGION 1..38: note = amidated human PTH 1-38
  MOD_RES 38: note = AMIDATION

SEQ ID NO: 108 - protein, 37 aa, synthetic construct; identical to SEQ ID NO: 48
  REGION 1..37: note = amidated human PTH 1-37
  MOD_RES 37: note = AMIDATION

SEQ ID NO: 109 - protein, 36 aa, synthetic construct; identical to SEQ ID NO: 49
  REGION 1..36: note = amidated human PTH 1-36
  MOD_RES 36: note = AMIDATION

SEQ ID NO: 110 - protein, 35 aa, synthetic construct; identical to SEQ ID NO: 50
  REGION 1..35: note = amidated human PTH 1-35
  MOD_RES 35: note = AMIDATION

SEQ ID NO: 111 - protein, 34 aa, synthetic construct; identical to SEQ ID NO: 51
  REGION 1..34: note = amidated human PTH 1-34
  MOD_RES 34: note = AMIDATION

SEQ ID NO: 112 - protein, 33 aa, synthetic construct; identical to SEQ ID NO: 52
  REGION 1..33: note = amidated human PTH 1-33
  MOD_RES 33: note = AMIDATION

SEQ ID NO: 113 - protein, 32 aa, synthetic construct; identical to SEQ ID NO: 53
  REGION 1..32: note = amidated human PTH 1-32
  MOD_RES 32: note = AMIDATION

SEQ ID NO: 114 - protein, 31 aa, synthetic construct; identical to SEQ ID NO: 54
  REGION 1..31: note = amidated human PTH 1-31
  MOD_RES 31: note = AMIDATION

SEQ ID NO: 115 - protein, 30 aa, synthetic construct; identical to SEQ ID NO: 55
  REGION 1..30: note = amidated human PTH 1-30
  MOD_RES 30: note = AMIDATION

SEQ ID NO: 116 - protein, 29 aa, synthetic construct
  REGION 1..29: note = amidated human PTH 1-29
  MOD_RES 29: note = AMIDATION
SVSEIQLMHNLGKHLNSMERVEWLRKKLQ

SEQ ID NO: 117 - protein, 28 aa, synthetic construct
  REGION 1..28: note = amidated human PTH 1-28
  MOD_RES 28: note = AMIDATION
SVSEIQLMHNLGKHLNSMERVEWLRKKL

SEQ ID NO: 118 - protein, 27 aa, synthetic construct
  REGION 1..27: note = amidated human PTH 1-27
  MOD_RES 27: note = AMIDATION
SVSEIQLMHNLGKHLNSMERVEWLRKK

SEQ ID NO: 119 - protein, 26 aa, synthetic construct
  REGION 1..26: note = amidated human PTH 1-26
  MOD_RES 26: note = AMIDATION
SVSEIQLMHNLGKHLNSMERVEWLRK

SEQ ID NO: 120 - protein, 25 aa, synthetic construct
  REGION 1..25: note = amidated human PTH 1-25
  MOD_RES 25: note = AMIDATION
SVSEIQLMHNLGKHLNSMERVEWLR

SEQ ID NO: 121 - protein, 141 aa, Homo sapiens
AVSEHQLLHDKGKSIQDLRRRFFLHHLIAEIHTAEIRATSEVSPNSKPSPNTKNHPVRFGSDDEGRYLTQETNKVETYKEQPLKTPGKKKKGKPGKRKEQEKKKRRTRSAWLDSGVTGSGLEGDHLSDTSTTSLELDSRRH

SEQ ID NO: 122 - protein, 36 aa, synthetic construct
  REGION 1..36: note = Artificial random coil
AVAEIQLMHQRAKWIQDARRRAFLHKLIAEIHTAEI